European Patent Application EP 4 524 150 A1, published March 19, 2025. Title: 抗原短肽用于筛选治疗与HPV相关的疾病的药物中的用途及其筛选的TCR. Applicant: 广州医科大学. The sequence listing filed with the application follows.

SEQUENCE LISTING (46 sequences)

SEQ ID NO: 1 - protein, 9 aa, synthetic construct
IVCPICSQK

SEQ ID NO: 2 - protein, 7 aa, synthetic construct
TSDPSYG

SEQ ID NO: 3 - protein, 8 aa, synthetic construct
QGSYDQQN

SEQ ID NO: 4 - protein, 15 aa, synthetic construct
AMRIDAGGTSYGKLT

SEQ ID NO: 5 - protein, 5 aa, synthetic construct
LNHNV

SEQ ID NO: 6 - protein, 6 aa, synthetic construct
YYDKDF

SEQ ID NO: 7 - protein, 13 aa, synthetic construct
ATSRDRVNTGELF

SEQ ID NO: 8 - protein, 5 aa, synthetic construct
DSVNN

SEQ ID NO: 9 - protein, 5 aa, synthetic construct
IPSGT

SEQ ID NO: 10 - protein, 16 aa, synthetic construct
AVEGDNAGGTSYGKLT

SEQ ID NO: 11 - protein, 5 aa, synthetic construct
MNHEY

SEQ ID NO: 12 - protein, 6 aa, synthetic construct
SMNVEV

SEQ ID NO: 13 - protein, 11 aa, synthetic construct
ASSWSTSYGYT

SEQ ID NO: 14 - protein, 6 aa, synthetic construct
NYSPAY

SEQ ID NO: 15 - protein, 7 aa, synthetic construct
IRENEKE

SEQ ID NO: 16 - protein, 9 aa, synthetic construct
ALAGYQKVT

SEQ ID NO: 17 - protein, 6 aa, synthetic construct
GTSNPN

SEQ ID NO: 18 - protein, 5 aa, synthetic construct
SVGIG

SEQ ID NO: 19 - protein, 12 aa, synthetic construct
AWSLRTSGSEQF

SEQ ID NO: 20 - protein, 20 aa, synthetic construct
MSLSSLLKVVTASLWLGPGI

SEQ ID NO: 21 - protein, 19 aa, synthetic construct
MGPGLLHWMALCLLGTGHG

SEQ ID NO: 22 - protein, 20 aa, synthetic construct
MKRILGALLGLLSAQVCCVR

SEQ ID NO: 23 - protein, 19 aa, synthetic construct
MGPQLLGYVVLCLLGAGPL

SEQ ID NO: 24 - protein, 20 aa, synthetic construct
MESFLGGVLLILWLQVDWVK

SEQ ID NO: 25 - protein, 17 aa, synthetic construct
MLCSLLALLLGTFFGVR

SEQ ID NO: 26 - protein, 139 aa, synthetic construct
MSLSSLLKVVTASLWLGPGIAQKITQTQPGMFVQEKEAVTLDCTYDTSDPSYGLFWYKQPSSGEMIFLIYQGSYDQQNATEGRYSLNFQKARKSANLVISASQLGDSAMYFCAMRIDAGGTSYGKLTFGQGTILTVHPN

SEQ ID NO: 27 - protein, 133 aa, synthetic construct
MGPGLLHWMALCLLGTGHGDAMVIQNPRYQVTQFGKPVTLSCSQTLNHNVMYWYQQKSSQAPKLLFHYYDKDFNNEADTPDNFQSRRPNTSFCFLDIRSPGLGDAAMYLCATSRDRVNTGELFFGEGSRLTVL

SEQ ID NO: 28 - protein, 135 aa, synthetic construct
MKRILGALLGLLSAQVCCVRGIQVEQSPPDLILQEGANSTLRCNFSDSVNNLQWFHQNPWGQLINLFYIPSGTKQNGRLSATTVATERYSLLYISSSQTTDSGVYFCAVEGDNAGGTSYGKLTFGQGTILTVHPN

SEQ ID NO: 29 - protein, 131 aa, synthetic construct
MGPQLLGYVVLCLLGAGPLEAQVTQNPRYLITVTGKKLTVTCSQNMNHEYMSWYRQDPGLGLRQIYYSMNVEVTDKGDVPEGYKVSRKEKRNFPLILESPSPNQTSLYFCASSWSTSYGYTFGSGTRLTIV

SEQ ID NO: 30 - protein, 131 aa, synthetic construct
MESFLGGVLLILWLQVDWVKSQKIEQNSEALNIQEGKTATLTCNYTNYSPAYLQWYRQDPGRGPVFLLLIRENEKEKRKERLKVTFDTTLKQSLFHITASQPADSATYLCALAGYQKVTFGTGTKLQVIPN

SEQ ID NO: 31 - protein, 130 aa, synthetic construct
MLCSLLALLLGTFFGVRSQTIHQWPATLVQPVGSPLSLECTVEGTSNPNLYWYRQAAGRGLQLLFYSVGIGQISSEVPQNLSASRPQDRQFILSSKKLLLSDSGFYLCAWSLRTSGSEQFFGPGTRLTVL

SEQ ID NO: 32 - protein, 136 aa, synthetic construct
IQNPEPAVYQLKDPRSQDSTLCLFTDFDSQINVPKTMESGTFITDKCVLDMKAMDSKSNGAIAWSNQTSFTCQDIFKETNATYPSSDVPCDATLTEKSFETDMNLNFQNLSVMGLRILLLKVAGFNLLMTLRLWSS

SEQ ID NO: 33 - protein, 173 aa, synthetic construct
EDLRNVTPPKVSLFEPSKAEIANKQKATLVCLARGFFPDHVELSWWVNGKEVHSGVCTDPQAYKESNYSYCLSSRLRVSATFWHNPRNHFRCQVQFHGLSEEDKWPEGSPKPVTQNISAEAWGRADCGITSASYHQGVLSATILYEILLGKATLYAVLVSGLVLMAMVKKKNS

SEQ ID NO: 34 - DNA, 825 bp, synthetic construct
  source 1..825: mol_type = other DNA
atgtcactttctagcctgctgaaggtggtcacagcttcactgtggctaggacctggcattgcccagaagataactcaaacccaaccaggaatgttcgtgcaggaaaaggaggctgtgactctggactgcacatatgacaccagtgatccaagttatggtctattctggtacaagcagcccagcagtggggaaatgatttttcttatttatcaggggtcttatgaccagcaaaatgcaacagaaggtcgctactcattgaatttccagaaggcaagaaaatccgccaaccttgtcatctccgcttcacaactgggggactcagcaatgtacttctgtgcaatgagaattgatgctggtggtactagctatggaaagctgacatttggacaagggaccatcttgactgtccatccaaatatccagaatccagagcccgccgtgtatcagctgaaggacccaaggagccaggattccaccctgtgcctgttcacagactttgatagccagatcaacgtgcccaagaccatggagtccggcaccttcatcacagacaagtgcgtgctggatatgaaggccatggactctaagagcaacggcgccatcgcctggagcaatcagacctccttcacatgccaggatatctttaaggagaccaatgccacatatccttcctctgacgtgccatgtgatgccaccctgacagagaagtccttcgagaccgacatgaacctgaattttcagaacctgtctgtgatgggcctgcgcatcctgctgctgaaggtggccggcttcaatctgctgatgaccctgaggctgtggagctcc

SEQ ID NO: 35 - DNA, 918 bp, synthetic construct
  source 1..918: mol_type = other DNA
atgggtcctgggcttctccactggatggccctttgtctccttggaacaggtcatggggatgccatggtcatccagaacccaagataccaggttacccagtttggaaagccagtgaccctgagttgttctcagactttgaaccataacgtcatgtactggtaccagcagaagtcaagtcaggccccaaagctgctgttccactactatgacaaagattttaacaatgaagcagacacccctgataacttccaatccaggaggccgaacacttctttctgctttcttgacatccgctcaccaggcctgggggacgcagccatgtacctgtgtgccaccagcagagatagggtcaacaccggggagctgttttttggagaaggctctaggctgaccgtactggaggatctgaggaacgtgacaccccctaaggtgtctctgttcgagcccagcaaggccgagatcgccaataagcagaaggccaccctggtgtgcctggcaaggggcttctttcctgatcacgtggagctgtcttggtgggtgaacggcaaggaggtgcacagcggcgtgtgcaccgacccacaggcctacaaggagtccaattactcttattgtctgagctcccggctgagagtgtccgccacattttggcacaaccctagaaatcacttcaggtgccaggtgcagtttcacggcctgagcgaggaggataagtggccagagggatccccaaagcctgtgacccagaacatctctgccgaggcatggggaagggcagactgtggaatcacatccgcctcttatcaccagggcgtgctgagcgccaccatcctgtacgagatcctgctgggcaaggccacactgtatgccgtgctggtgagcggcctggtgctgatggccatggtgaagaagaagaactcc

SEQ ID NO: 36 - DNA, 813 bp, synthetic construct
  source 1..813: mol_type = other DNA
atgaagaggatattgggagctctgctggggctcttgagtgcccaggtttgctgtgtgagaggaatacaagtggagcagagtcctccagacctgattctccaggagggagccaattccacgctgcggtgcaatttttctgactctgtgaacaatttgcagtggtttcatcaaaacccttggggacagctcatcaacctgttttacattccctcagggacaaaacagaatggaagattaagcgccacgactgtcgctacggaacgctacagcttattgtacatttcctcttcccagaccacagactcaggcgtttatttctgtgctgtggagggggataatgctggtggtactagctatggaaagctgacatttggacaagggaccatcttgactgtccatccaaatatccagaatccagagcccgccgtgtatcagctgaaggacccaaggagccaggattccaccctgtgcctgttcacagactttgatagccagatcaacgtgcccaagaccatggagtccggcaccttcatcacagacaagtgcgtgctggatatgaaggccatggactctaagagcaacggcgccatcgcctggagcaatcagacctccttcacatgccaggatatctttaaggagaccaatgccacatatccttcctctgacgtgccatgtgatgccaccctgacagagaagtccttcgagaccgacatgaacctgaattttcagaacctgtctgtgatgggcctgcgcatcctgctgctgaaggtggccggcttcaatctgctgatgaccctgaggctgtggagctcc

SEQ ID NO: 37 - DNA, 912 bp, synthetic construct
  source 1..912: mol_type = other DNA
atgggcccccagctccttggctatgtggtcctttgccttctaggagcaggccccctggaagcccaagtgacccagaacccaagatacctcatcacagtgactggaaagaagttaacagtgacttgttctcagaatatgaaccatgagtatatgtcctggtatcgacaagacccagggctgggcttaaggcagatctactattcaatgaatgttgaggtgactgataagggagatgttcctgaagggtacaaagtctctcgaaaagagaagaggaatttccccctgatcctggagtcgcccagccccaaccagacctctctgtacttctgtgccagcagttggtcgacctcctatggctacaccttcggttcggggaccaggttaaccattgtagaggatctgaggaacgtgacaccccctaaggtgtctctgttcgagcccagcaaggccgagatcgccaataagcagaaggccaccctggtgtgcctggcaaggggcttctttcctgatcacgtggagctgtcttggtgggtgaacggcaaggaggtgcacagcggcgtgtgcaccgacccacaggcctacaaggagtccaattactcttattgtctgagctcccggctgagagtgtccgccacattttggcacaaccctagaaatcacttcaggtgccaggtgcagtttcacggcctgagcgaggaggataagtggccagagggatccccaaagcctgtgacccagaacatctctgccgaggcatggggaagggcagactgtggaatcacatccgcctcttatcaccagggcgtgctgagcgccaccatcctgtacgagatcctgctgggcaaggccacactgtatgccgtgctggtgagcggcctggtgctgatggccatggtgaagaagaagaactcc

SEQ ID NO: 38 - DNA, 801 bp, synthetic construct
  source 1..801: mol_type = other DNA
atggagtcattcctgggaggtgttttgctgattttgtggcttcaagtggactgggtgaagagccaaaagatagaacagaattccgaggccctgaacattcaggagggtaaaacggccaccctgacctgcaactatacaaactattccccagcatacttacagtggtaccgacaagatccaggaagaggccctgttttcttgctactcatacgtgaaaatgagaaagaaaaaaggaaagaaagactgaaggtcacctttgataccacccttaaacagagtttgtttcatatcacagcctcccagcctgcagactcagctacctacctctgtgctctcgcgggttaccagaaagttacctttggaactggaacaaagctccaagtcatcccaaatatccagaatccagagcccgccgtgtatcagctgaaggacccaaggagccaggattccaccctgtgcctgttcacagactttgatagccagatcaacgtgcccaagaccatggagtccggcaccttcatcacagacaagtgcgtgctggatatgaaggccatggactctaagagcaacggcgccatcgcctggagcaatcagacctccttcacatgccaggatatctttaaggagaccaatgccacatatccttcctctgacgtgccatgtgatgccaccctgacagagaagtccttcgagaccgacatgaacctgaattttcagaacctgtctgtgatgggcctgcgcatcctgctgctgaaggtggccggcttcaatctgctgatgaccctgaggctgtggagctcc

SEQ ID NO: 39 - DNA, 909 bp, synthetic construct
  source 1..909: mol_type = other DNA
atgctctgctctctccttgcccttctcctgggcactttctttggggtcagatctcagactattcatcaatggccagcgaccctggtgcagcctgtgggcagcccgctctctctggagtgcactgtggagggaacatcaaaccccaacctatactggtaccgacaggctgcaggcaggggcctccagctgctcttctactccgttggtattggccagatcagctctgaggtgccccagaatctctcagcctccagaccccaggaccggcagttcatcctgagttctaagaagctccttctcagtgactctggcttctatctctgtgcctggagtctccggactagcgggagcgagcagttcttcgggccagggacacggctcaccgtgctagaggatctgaggaacgtgacaccccctaaggtgtctctgttcgagcccagcaaggccgagatcgccaataagcagaaggccaccctggtgtgcctggcaaggggcttctttcctgatcacgtggagctgtcttggtgggtgaacggcaaggaggtgcacagcggcgtgtgcaccgacccacaggcctacaaggagtccaattactcttattgtctgagctcccggctgagagtgtccgccacattttggcacaaccctagaaatcacttcaggtgccaggtgcagtttcacggcctgagcgaggaggataagtggccagagggatccccaaagcctgtgacccagaacatctctgccgaggcatggggaagggcagactgtggaatcacatccgcctcttatcaccagggcgtgctgagcgccaccatcctgtacgagatcctgctgggcaaggccacactgtatgccgtgctggtgagcggcctggtgctgatggccatggtgaagaagaagaactcc

SEQ ID NO: 40 - protein, 367 aa, synthetic construct
MAVMAPRTLLLLLSGALALTQTWAGSHSMRYFYTSVSRPGRGEPRFIAVGYVDDTQFVRFDSDAASQRMEPRAPWIEQEGPEYWDQETRNVKAQSQTDRVDLGTLRGYYNQSEDGSHTIQIMYGCDVGPDGRFLRGYRQDAYDGKDYIALNEDLRSWTAADMAAQITKRKWEAAHAAEQQRAYLEGRCVEWLRRYLENGKETLQRTDPPKTHMTHHPISDHEATLRCWALGFYPAEITLTWQRDGEDQTQDTELVETRPAGDGTFQKWAAVVVPSGEEQRYTCHVQHEGLPKPLTLRWELSSQPTIPIVGIIAGLVLLGAVITGAVVAAVMWRRKSSDRKGGSYTQAASSDSAQGSDVSLTACKVSR

SEQ ID NO: 41 - DNA, 417 bp, synthetic construct
  source 1..417: mol_type = other DNA
atgtcactttctagcctgctgaaggtggtcacagcttcactgtggctaggacctggcattgcccagaagataactcaaacccaaccaggaatgttcgtgcaggaaaaggaggctgtgactctggactgcacatatgacaccagtgatccaagttatggtctattctggtacaagcagcccagcagtggggaaatgatttttcttatttatcaggggtcttatgaccagcaaaatgcaacagaaggtcgctactcattgaatttccagaaggcaagaaaatccgccaaccttgtcatctccgcttcacaactgggggactcagcaatgtacttctgtgcaatgagaattgatgctggtggtactagctatggaaagctgacatttggacaagggaccatcttgactgtccatccaaat

SEQ ID NO: 42 - DNA, 399 bp, synthetic construct
  source 1..399: mol_type = other DNA
atgggtcctgggcttctccactggatggccctttgtctccttggaacaggtcatggggatgccatggtcatccagaacccaagataccaggttacccagtttggaaagccagtgaccctgagttgttctcagactttgaaccataacgtcatgtactggtaccagcagaagtcaagtcaggccccaaagctgctgttccactactatgacaaagattttaacaatgaagcagacacccctgataacttccaatccaggaggccgaacacttctttctgctttcttgacatccgctcaccaggcctgggggacgcagccatgtacctgtgtgccaccagcagagatagggtcaacaccggggagctgttttttggagaaggctctaggctgaccgtactg

SEQ ID NO: 43 - DNA, 405 bp, synthetic construct
  source 1..405: mol_type = other DNA
atgaagaggatattgggagctctgctggggctcttgagtgcccaggtttgctgtgtgagaggaatacaagtggagcagagtcctccagacctgattctccaggagggagccaattccacgctgcggtgcaatttttctgactctgtgaacaatttgcagtggtttcatcaaaacccttggggacagctcatcaacctgttttacattccctcagggacaaaacagaatggaagattaagcgccacgactgtcgctacggaacgctacagcttattgtacatttcctcttcccagaccacagactcaggcgtttatttctgtgctgtggagggggataatgctggtggtactagctatggaaagctgacatttggacaagggaccatcttgactgtccatccaaat

SEQ ID NO: 44 - DNA, 393 bp, synthetic construct
  source 1..393: mol_type = other DNA
atgggcccccagctccttggctatgtggtcctttgccttctaggagcaggccccctggaagcccaagtgacccagaacccaagatacctcatcacagtgactggaaagaagttaacagtgacttgttctcagaatatgaaccatgagtatatgtcctggtatcgacaagacccagggctgggcttaaggcagatctactattcaatgaatgttgaggtgactgataagggagatgttcctgaagggtacaaagtctctcgaaaagagaagaggaatttccccctgatcctggagtcgcccagccccaaccagacctctctgtacttctgtgccagcagttggtcgacctcctatggctacaccttcggttcggggaccaggttaaccattgta

SEQ ID NO: 45 - DNA, 393 bp, synthetic construct
  source 1..393: mol_type = other DNA
atggagtcattcctgggaggtgttttgctgattttgtggcttcaagtggactgggtgaagagccaaaagatagaacagaattccgaggccctgaacattcaggagggtaaaacggccaccctgacctgcaactatacaaactattccccagcatacttacagtggtaccgacaagatccaggaagaggccctgttttcttgctactcatacgtgaaaatgagaaagaaaaaaggaaagaaagactgaaggtcacctttgataccacccttaaacagagtttgtttcatatcacagcctcccagcctgcagactcagctacctacctctgtgctctcgcgggttaccagaaagttacctttggaactggaacaaagctccaagtcatcccaaat

SEQ ID NO: 46 - DNA, 390 bp, synthetic construct
  source 1..390: mol_type = other DNA
atgctctgctctctccttgcccttctcctgggcactttctttggggtcagatctcagactattcatcaatggccagcgaccctggtgcagcctgtgggcagcccgctctctctggagtgcactgtggagggaacatcaaaccccaacctatactggtaccgacaggctgcaggcaggggcctccagctgctcttctactccgttggtattggccagatcagctctgaggtgccccagaatctctcagcctccagaccccaggaccggcagttcatcctgagttctaagaagctccttctcagtgactctggcttctatctctgtgcctggagtctccggactagcgggagcgagcagttcttcgggccagggacacggctcaccgtgcta